European Patent Application EP 4 310 499 A1, published January 24, 2024. Title: Biological Detection Chip and Application Thereof. Applicant: Sunplus Technology Co. Ltd. Application EP. The sequence listing filed with the application follows.

SEQUENCE LISTING (15 sequences)

SEQ ID NO: 1 - DNA, 20 bp, synthetic construct
  source 1..20: mol_type = other DNA
  modified_base 8: mod_base = i
  modified_base 17: mod_base = i
cggcccanttccatccngag

SEQ ID NO: 2 - DNA, 23 bp, synthetic construct
  source 1..23: mol_type = other DNA
  modified_base 16: mod_base = i
cattcagctcgcatancgtcaag

SEQ ID NO: 3 - DNA, 19 bp, synthetic construct
  source 1..19: mol_type = other DNA
  modified_base 5: mod_base = i
  modified_base 12: mod_base = i
tgctncatttcntgacacc

SEQ ID NO: 4 - DNA, 18 bp, synthetic construct
  source 1..18: mol_type = other DNA
  modified_base 9: mod_base = i
  modified_base 12: mod_base = i
accttaagngcntatatc

SEQ ID NO: 5 - DNA, 19 bp, synthetic construct
  source 1..19: mol_type = other DNA
taccaacttcattgtggac

SEQ ID NO: 6 - DNA, 18 bp, synthetic construct
  source 1..18: mol_type = other DNA
acccagcaactggcacag

SEQ ID NO: 7 - DNA, 18 bp, synthetic construct
  source 1..18: mol_type = other DNA
  modified_base 14: mod_base = i
tggcccctgcccancacg

SEQ ID NO: 8 - DNA, 21 bp, synthetic construct
  source 1..21: mol_type = other DNA
tcgccctaattgaataggtga

SEQ ID NO: 9 - DNA, 18 bp, synthetic construct
  source 1..18: mol_type = other DNA
gcctggttcgargacctc

SEQ ID NO: 10 - DNA, 20 bp, synthetic construct
  source 1..20: mol_type = other DNA
tacgggcgygctcgtgacca

SEQ ID NO: 11 - DNA, 19 bp, synthetic construct
  source 1..19: mol_type = other DNA
ctggcacagaattgcaggt

SEQ ID NO: 12 - DNA, 20 bp, synthetic construct
  source 1..20: mol_type = other DNA
tgaaaaggtactgcgttccc

SEQ ID NO: 13 - DNA, 18 bp, synthetic construct
  source 1..18: mol_type = other DNA
ccatagcccagcagccaa

SEQ ID NO: 14 - DNA, 29 bp, synthetic construct
  source 1..29: mol_type = other DNA
tccttcttgcactgacattaccactggct

SEQ ID NO: 15 - DNA, 29 bp, synthetic construct
  source 1..29: mol_type = other DNA
agccagtggtaatgtcagtgcaagaagga